European Patent Application EP 4 763 992 A1, published June 24, 2026. Title: Methods and kits for isolating a target nucleic acid by in-gel affinity electrophoresis. Applicant: Johannes Gutenberg-Universität Mainz. Application EP. The sequence listing filed with the application follows.

SEQUENCE LISTING (24 sequences)

SEQ ID NO: 1 - DNA, 80 bp, synthetic construct
  source 1..80: mol_type = other DNA
ttttttttttttttttttttagcgcttatgttttttttttttttttttttagcgcttatgtttttttttttttttttttt

SEQ ID NO: 2 - DNA, 80 bp, synthetic construct; identical to SEQ ID NO: 1
  source 1..80: mol_type = other DNA

SEQ ID NO: 3 - DNA, 80 bp, synthetic construct; identical to SEQ ID NO: 1
  source 1..80: mol_type = other DNA

SEQ ID NO: 4 - DNA, 79 bp, synthetic construct
  source 1..79: mol_type = other DNA
ggcaccaccccggtgaacagctcctcgcccttgctcaccatggttgtggaaggggggtgtttggtgcctgggttacata

SEQ ID NO: 5 - DNA, 44 bp, synthetic construct
  source 1..44: mol_type = other DNA
cgctcgacgtacgctcgacgtacgctcgacgtacgctcgacgta

SEQ ID NO: 6 - DNA, 86 bp, synthetic construct
  source 1..86: mol_type = other DNA
aaaaaaaaaaaaaaaaaaaaaacataagcgctaaaaaaaaaaaaaaaaaaaaggctgctcacggggtctcctctaacctctagtcc

SEQ ID NO: 7 - DNA, 79 bp, synthetic construct
  source 1..79: mol_type = other DNA
tacgtcgagcgtacgtcgagcgtacgtcgagcgtacgtcgagcgacgaacggtcgggggtctcctctaacctctagtcc

SEQ ID NO: 8 - DNA, 48 bp, synthetic construct
  source 1..48: mol_type = other DNA
ctaggaacttctctaggaacttctctaggaacttctctaggaacttct

SEQ ID NO: 9 - DNA, 82 bp, synthetic construct
  source 1..82: mol_type = other DNA
agaagttcctagagaagttcctagagaagttcctagccgtgaccctagggtgagggggggattcgaacccccgatacgttgc

SEQ ID NO: 10 - DNA, 82 bp, synthetic construct
  source 1..82: mol_type = other DNA
agaagttcctagagaagttcctagagaagttcctagccgtgaccctaggcgaggggggggacttgaacccccacgtccgtaa

SEQ ID NO: 11 - DNA, 36 bp, synthetic construct
  source 1..36: mol_type = other DNA
taggacactcaataggacactcaataggacactcaa

SEQ ID NO: 12 - DNA, 82 bp, synthetic construct
  source 1..82: mol_type = other DNA
ttgagtgtcctattgagtgtcctattgagtgtcctaccgtgaccctagggtgagggggggattcgaacccccgatacgttgc

SEQ ID NO: 13 - DNA, 82 bp, synthetic construct
  source 1..82: mol_type = other DNA
ttgagtgtcctattgagtgtcctattgagtgtcctaccgtgaccctaggcgaggggggggacttgaacccccacgtccgtaa

SEQ ID NO: 14 - DNA, 80 bp, synthetic construct
  source 1..80: mol_type = other DNA
aaaaaaaaaaaaaaaaaaaaaacataagcgctaaaaaaaaaaaaaaaaaaaaggctgctcacttgctcccatggttgtgg

SEQ ID NO: 15 - DNA, 36 bp, synthetic construct
  source 1..36: mol_type = other DNA
ccacaaccatgggagcaaccacaaccatgggagcaa

SEQ ID NO: 16 - DNA, 31 bp, synthetic construct
  source 1..31: mol_type = other DNA
ggactagccttcagagttgctcccatggttg

SEQ ID NO: 17 - DNA, 30 bp, synthetic construct
  source 1..30: mol_type = other DNA
ctctgaaggctagtctatgcgcatacgact

SEQ ID NO: 18 - DNA, 13 bp, synthetic construct
  source 1..13: mol_type = other DNA
actcgacagatac

SEQ ID NO: 19 - DNA, 40 bp, synthetic construct
  source 1..40: mol_type = other DNA
aaaaaaaaaaaaaaaaaaaaaaaaaaaaaaaaaaaaaaaa

SEQ ID NO: 20 - DNA, 20 bp, synthetic construct
  source 1..20: mol_type = other DNA
atgggagaccgcctgggaat

SEQ ID NO: 21 - DNA, 25 bp, synthetic construct
  source 1..25: mol_type = other DNA
ggacacattgatcatcgacacttcg

SEQ ID NO: 22 - DNA, 34 bp, synthetic construct
  source 1..34: mol_type = other DNA
cacccgagattgagcaataacaggtctgtgatgc

SEQ ID NO: 23 - DNA, 40 bp, synthetic construct
  source 1..40: mol_type = other DNA
aagtggcgttcagccacccgagattgagcaataacaggtc

SEQ ID NO: 24 - DNA, 4520 bp, synthetic construct
  source 1..4520: mol_type = other DNA
ggtaccgagctcttacgcgtgctagcccgggctcgagatctgcgatctaagtaagctttaatacgactcactataggtagaagtcaggtcggattaagccatagtacggaaaaaactatgctacctgtgagccccgtccaaggacgttaaaagaagtcaggccattacaaatgccatagcttgagtaaactgtgcagcctgtagctccacctgagaaggtgtaaaaaatctgggaggccacaaaccatggaagctgtacgcatggcgtagtggactagcggttagaggagacccctcccttacaaatcgcagcaacaatgggggcccaaggtgagatgaagctgtagtctcactggaaggactagaggttagaggagacccccccaaaacaaaaaacagcatattgacgctgggaaagaccagagatcctgctgtctcctcagcatcattccaggcacagaacgccagaaaatggaatggtgctgttgaatcaacaggttctctagaatgacttcgaaagtttatgatccagaacaaaggaaacggatgataactggtccgcagtggtgggccagatgtaaacaaatgaatgttcttgattcatttattaattattatgattcagaaaaacatgcagaaaatgctgttatttttttacatggtaacgcggcctcttcttatttatggcgacatgttgtgccacatattgagccagtagcgcggtgtattataccagaccttattggtatgggcaaatcaggcaaatctggtaatggttcttataggttacttgatcattacaaatatcttactgcatggtttgaacttcttaatttaccaaagaagatcatttttgtcggccatgattggggtgcttgtttggcatttcattatagctatgagcatcaagataagatcaaagcaatagttcacgctgaaagtgtagtagatgtgattgaatcatgggatgaatggcctgatattgaagaagatattgcgttgatcaaatctgaagaaggagaaaaaatggttttggagaataacttcttcgtggaaaccatgttgccatcaaaaatcatgagaaagttagaaccagaagaatttgcagcatatcttgaaccattcaaagagaaaggtgaagttcgtcgtccaacattatcatggcctcgtgaaatcccgttagtaaaaggtggtaaacctgacgttgtacaaattgttaggaattataatgcttatctacgtgcaagtgatgatttaccaaaaatgtttattgaatcggacccaggattcttttccaatgctattgttgaaggtgccaagaagtttcctaatactgaatttgtcaaagtaaaaggtcttcatttttcgcaagaagatgcacctgatgaaatgggaaaatatatcaaatcgttcgttgagcgagttctcaaaaatgaacaataatctagagtcggggcggccggccgcttcgagcagacatgataagatacattgatgagtttggacaaaccacaactagaatgcagtgaaaaaaatgctttatttgtgaaatttgtgatgctattgctttatttgtaaccattataagctgcaataaacaagttaacaacaacaattgcattcattttatgtttcaggttcagggggaggtgtgggaggttttttaaagcaagtaaaacctctacaaatgtggtaaaatcgataaggatccgtcgaccgatgcccttgagagccttcaacccagtcagctccttccggtgggcgcggggcatgactatcgtcgccgcacttatgactgtcttctttatcatgcaactcgtaggacaggtgccggcagcgctcttccgcttcctcgctcactgactcgctgcgctcggtcgttcggctgcggcgagcggtatcagctcactcaaaggcggtaatacggttatccacagaatcaggggataacgcaggaaagaacatgtgagcaaaaggccagcaaaaggccaggaaccgtaaaaaggccgcgttgctggcgtttttccataggctccgcccccctgacgagcatcacaaaaatcgacgctcaagtcagaggtggcgaaacccgacaggactataaagataccaggcgtttccccctggaagctccctcgtgcgctctcctgttccgaccctgccgcttaccggatacctgtccgcctttctcccttcgggaagcgtggcgctttctcaatgctcacgctgtaggtatctcagttcggtgtaggtcgttcgctccaagctgggctgtgtgcacgaaccccccgttcagcccgaccgctgcgccttatccggtaactatcgtcttgagtccaacccggtaagacacgacttatcgccactggcagcagccactggtaacaggattagcagagcgaggtatgtaggcggtgctacagagttcttgaagtggtggcctaactacggctacactagaaggacagtatttggtatctgcgctctgctgaagccagttaccttcggaaaaagagttggtagctcttgatccggcaaacaaaccaccgctggtagcggtggtttttttgtttgcaagcagcagattacgcgcagaaaaaaaggatctcaagaagatcctttgatcttttctacggggtctgacgctcagtggaacgaaaactcacgttaagggattttggtcatgagattatcaaaaaggatcttcacctagatccttttaaattaaaaatgaagttttaaatcaatctaaagtatatatgagtaaacttggtctgacagttaccaatgcttaatcagtgaggcacctatctcagcgatctgtctatttcgttcatccatagttgcctgactccccgtcgtgtagataactacgatacgggagggcttaccatctggccccagtgctgcaatgataccgcgagacccacgctcaccggctccagatttatcagcaataaaccagccagccggaagggccgagcgcagaagtggtcctgcaactttatccgcctccatccagtctattaattgttgccgggaagctagagtaagtagttcgccagttaatagtttgcgcaacgttgttgccattgctacaggcatcgtggtgtcacgctcgtcgtttggtatggcttcattcagctccggttcccaacgatcaaggcgagttacatgatcccccatgttgtgcaaaaaagcggttagctccttcggtcctccgatcgttgtcagaagtaagttggccgcagtgttatcactcatggttatggcagcactgcataattctcttactgtcatgccatccgtaagatgcttttctgtgactggtgagtactcaaccaagtcattctgagaatagtgtatgcggcgaccgagttgctcttgcccggcgtcaatacgggataataccgcgccacatagcagaactttaaaagtgctcatcattggaaaacgttcttcggggcgaaaactctcaaggatcttaccgctgttgagatccagttcgatgtaacccactcgtgcacccaactgatcttcagcatcttttactttcaccagcgtttctgggtgagcaaaaacaggaaggcaaaatgccgcaaaaaagggaataagggcgacacggaaatgttgaatactcatactcttcctttttcaatattattgaagcatttatcagggttattgtctcatgagcggatacatatttgaatgtatttagaaaaataaacaaataggggttccgcgcacatttccccgaaaagtgccacctgacgcgccctgtagcggcgcattaagcgcggcgggtgtggtggttacgcgcagcgtgaccgctacacttgccagcgccctagcgcccgctcctttcgctttcttcccttcctttctcgccacgttcgccggctttccccgtcaagctctaaatcgggggctccctttagggttccgatttagtgctttacggcacctcgaccccaaaaaacttgattagggtgatggttcacgtagtgggccatcgccctgatagacggtttttcgccctttgacgttggagtccacgttctttaatagtggactcttgttccaaactggaacaacactcaaccctatctcggtctattcttttgatttataagggattttgccgatttcggcctattggttaaaaaatgagctgatttaacaaaaatttaacgcgaattttaacaaaatattaacgtttacaatttcccattcgccattcaggctgcgcaactgttgggaagggcgatcggtgcgggcctcttcgctattacgccagcccaagctaccatgataagtaagtaatattaaggtacgggaggtacttggagcggccgcaataaaatatctttattttcattacatctgtgtgttggttttttgtgtgaatcgatagtactaacatacgctctccatcaaaacaaaacgaaacaaaacaaactagcaaaataggctgtccccagtgcaagtgcaggtgccagaacatttctctatcgata